European Patent Specification EP 3 461 843 B1, published September 6, 2023. Title: ANTI-CD19 ANTIBODY HAVING ADCC AND CDC FUNCTIONS AND IMPROVED GLYCOSYLATION PROFILE. Applicant: IDD BIOTECH (INTERNATIONAL - DRUG - DEVELOPMENT - BIOTECH). Application EP 10/305796. The sequence listing filed with the application follows.

SEQUENCE LISTING (36 sequences)

SEQ ID NO: 1 - protein, 330 aa, artificial sequence
  Fc34
ASTKGPSVFPLAPSSKSTSGGTAALGCLVKDYFPEPVTVSWNSGALTSGVHTFPAVLQSSGLYSLSSVVTVPSSSLGTQTYICNVNHKPSNTKVDKKVEPKSCDKTHTCPPCPAPELLGGPSVFLLPPKPKDTLMISRTPEVTCVVVDVSHEDPEVKFNWYVDGVEVHNAKTKPPEEQYNSTLRVVSLLTVLHQDWLNGKEYKCKVSNAALPAPIEKTISKAKGQPREPQVYTLPPSRDELTKNQVSLTCLVKGFYPSDIAVEWESNGQPENNYKTTPLVLDSDGSFFLYSKLTVDKSRWQQGNVFSCSVMHEALHNHYTQKSLSLSPGK

SEQ ID NO: 2 - DNA, 993 bp, artificial sequence
  Fc34
gcctccaccaagggcccatcggtcttccccctggcaccctcctccaagagcacctctgggggcacagcggccctgggctgcctggtcaaggactacttccccgaaccggtgacggtgtcgtggaactcaggcgccctgaccagcggcgtgcacaccttcccggctgtcctacagtcctcaggactctactccctcagcagcgtcgtgaccgtgccctccagcagcttgggcacccagacctacatctgcaacgtgaatcacaagcccagcaacaccaaggtggacaagaaagttgagcccaaatcttgtgacaaaactcacacatgcccaccgtgcccagcacctgaactcctggggggaccgtcagtcttcctcttacccccaaaacccaaggacaccctcatgatctcccggacccctgaggtcacatgcgtggtggtggacgtgagccacgaagaccctgaggtcaagttcaactggtacgtggacggcgtggaggtgcataatgccaagacaaagccgccggaggagcagtacaacagcacgctccgtgtggtcagcctcctcaccgtcctgcaccaggactggctgaatggcaaggagtacaagtgcaaggtctccaacgcagccctcccagcccccatcgagaaaaccatctccaaagccaaagggcagccccgagaaccacaggtgtacaccctgcccccatcccgggatgagctgaccaagaaccaggtcagcctgacctgcctggtcaaaggcttctatcccagcgacatcgccgtggagtgggagagcaatgggcagccggagaacaactacaagaccacgcctctcgtgctggactccgacggctccttcttcctctacagcaagctcaccgtggacaagagcaggtggcagcaggggaacgtcttctcatgctccgtgatgcatgaggctctgcacaaccactacacgcagaagagcctctccctgtctccgggtaaatga

SEQ ID NO: 3 - protein, 330 aa, artificial sequence
  Fc24
ASTKGPSVFPLAPSSKSTSGGTAALGCLVKDYFPEPVTVSWNSGALTSGVHTFPAVLQSSGLYSLSSVVTVPSSSLGTQTYICNVNHKPSNTKVDKKVEPKSCDKTHTCPPCPAPELLGGPSVFLLPPKPKDTLMISRTPEVTCVVVDVSHEDPEVKFNWYVDGVEVHNAKTKPPEEQYNSTLRVVSLLTVLHQDWLNGKEYKCKVSNAALPAPIAKTISKAKGQPREPQVYTLPPSRDELTKNQVSLTCLVKGFYPSDIAVEWESNGQPENNYKTTPLVLDSDGSFFLYSKLTVDKSRWQQGNVFSCSVMHEALHNHYTQKSLSLSPGK

SEQ ID NO: 4 - DNA, 993 bp, artificial sequence
  Fc24
gcctccaccaagggcccatcggtcttccccctggcaccctcctccaagagcacctctgggggcacagcggccctgggctgcctggtcaaggactacttccccgaaccggtgacggtgtcgtggaactcaggcgccctgaccagcggcgtgcacaccttcccggctgtcctacagtcctcaggactctactccctcagcagcgtcgtgaccgtgccctccagcagcttgggcacccagacctacatctgcaacgtgaatcacaagcccagcaacaccaaggtggacaagaaagttgagcccaaatcttgtgacaaaactcacacatgcccaccgtgcccagcacctgaactcctggggggaccgtcagtcttcctcttacccccaaaacccaaggacaccctcatgatctcccggacccctgaggtcacatgcgtggtggtggacgtgagccacgaagaccctgaggtcaagttcaactggtacgtggacggcgtggaggtgcataatgccaagacaaagccgccggaggagcagtacaacagcacgctccgtgtggtcagcctcctcaccgtcctgcaccaggactggctgaatggcaaggagtacaagtgcaaggtctccaacgcagccctcccagcccccatcgcgaaaaccatctccaaagccaaagggcagccccgagaaccacaggtgtacaccctgcccccatcccgggatgagctgaccaagaaccaggtcagcctgacctgcctggtcaaaggcttctatcccagcgacatcgccgtggagtgggagagcaatgggcagccggagaacaactacaagaccacgcctctcgtgctggactccgacggctccttcttcctctacagcaagctcaccgtggacaagagcaggtggcagcaggggaacgtcttctcatgctccgtgatgcatgaggctctgcacaaccactacacgcagaagagcctctccctgtctccgggtaaatga

SEQ ID NO: 5 - protein, 8 aa, artificial sequence
  peptide
GYAFSSYW

SEQ ID NO: 6 - protein, 8 aa, artificial sequence
  peptide
IYPGDGDT

SEQ ID NO: 7 - protein, 14 aa, artificial sequence
  peptide
ARSITTVVGCAMDY

SEQ ID NO: 8 - protein, 6 aa, artificial sequence
  peptide
DHINNW

SEQ ID NO: 9 - protein, 3 aa, artificial sequence
  peptide
GAT

SEQ ID NO: 10 - protein, 9 aa, artificial sequence
  peptide
QQSWNTPWT

SEQ ID NO: 11 - protein, 5 aa, artificial sequence
  peptide
SYWVN

SEQ ID NO: 12 - protein, 17 aa, artificial sequence
  peptide
QIYPGDGDTNYNGKFKG

SEQ ID NO: 13 - protein, 12 aa, artificial sequence
  peptide
SITTVVGCAMDY

SEQ ID NO: 14 - protein, 11 aa, artificial sequence
  peptide
KASDHINNWLA

SEQ ID NO: 15 - protein, 7 aa, artificial sequence
  peptide
GATTLET

SEQ ID NO: 16 - protein, 4 aa, artificial sequence
  peptide
SSYW

SEQ ID NO: 17 - protein, 8 aa, artificial sequence
  peptide
GYTFTSYV

SEQ ID NO: 18 - protein, 8 aa, artificial sequence
  peptide
VNPYNDGT

SEQ ID NO: 19 - protein, 14 aa, artificial sequence
  peptide
ARGPYYYGSSPFDY

SEQ ID NO: 20 - protein, 11 aa, artificial sequence
  peptide
QSLENSNGNTY

SEQ ID NO: 21 - protein, 3 aa, artificial sequence
  peptide
RVS

SEQ ID NO: 22 - protein, 9 aa, artificial sequence
  peptide
LQVTHVPPT

SEQ ID NO: 23 - protein, 5 aa, artificial sequence
  peptide
SYVMH

SEQ ID NO: 24 - protein, 17 aa, artificial sequence
  peptide
YVNPYNDGTKYNEKFKG

SEQ ID NO: 25 - protein, 12 aa, artificial sequence
  peptide
GPYYYGSSPFDY

SEQ ID NO: 26 - protein, 16 aa, artificial sequence
  peptide
RSSQSLENSNGNTYLN

SEQ ID NO: 27 - protein, 7 aa, artificial sequence
  peptide
RVSNRFS

SEQ ID NO: 28 - protein, 4 aa, artificial sequence
  peptide
TSYV

SEQ ID NO: 29 - protein, 121 aa, artificial sequence
  protein
QVQLQQSGAELVRPGSSVKISCKASGYAFSSYWVNWMKQRPGQGLEWIGQIYPGDGDTNYNGKFKGRATVTADKSSSTSYMQFSSLTSEDSAVYFCARSITTVVGCAMDYWGQGTSVTVSS

SEQ ID NO: 30 - DNA, 363 bp, artificial sequence
  DNA
caggtccagctgcagcagtctggggctgaactggtgaggcctgggtcctcagtgaagatttcctgtaaggcttctggctatgcattcagtagctactgggtgaactggatgaagcagaggcctggacagggacttgagtggattggacagatttaccctggagatggtgatactaattacaatggaaagttcaagggtcgagccacagtgactgcagacaaatcctccagcacatcctacatgcagttcagcagcctaacatctgaggactctgcggtctatttctgtgcaagatctattactacggtggtaggctgtgctatggactactggggtcaaggaacctcggtcaccgtctcctca

SEQ ID NO: 31 - protein, 103 aa, artificial sequence
  peptide
DIQMTQSSAYLSVSLGGRVTITCKASDHINNWLAWYQHKPGNAPRLLISGATTLETGVPSRFSGSGSGKDYTLSITSLQTEDVATYYCQQSWNTPWTFGGGTK

SEQ ID NO: 32 - DNA, 309 bp, artificial sequence
  DNA
gacattcagatgacccagtcttctgcctacctgtctgtatctctaggaggcagggtcaccattacttgcaaggcaagtgaccacattaataattggttagcctggtatcaacataaaccaggaaatgctcctaggctcttaatatctggtgcaaccactttggaaactggggttccttcaagattcagtggcagtggatctggaaaggattacactctcagcattaccagtcttcagactgaagatgttgctacttattactgtcaacagtcttggaatactccgtggacgttcggtggaggcaccaag

SEQ ID NO: 33 - protein, 120 aa, artificial sequence
  protein
EVQLQQSGPELVKPGASVKMSCKASGYTFTSYVMHWVKQKPGQGLEWIGYVNPYNDGTKYNEKFKGKATLTSDKSSSTAYMELSSLTSEDSAVYYCARGPYYYGSSPFDYWGQGQVTVSS

SEQ ID NO: 34 - DNA, 360 bp, artificial sequence
  DNA
gaggttcagctgcaacagtctggacctgagctggtaaagcctggggcttcagtgaagatgtcctgcaaggcttctggatacacattcactagctatgttatgcactgggtgaagcagaagcctgggcagggccttgagtggattggatatgttaatccttacaatgatggtactaagtacaatgagaagttcaaaggcaaggccacactgacttcagacaaatcctccagcacagcctacatggagctcagcagcctgacctctgaggactctgcggtctattactgtgcaagagggccttattactacggtagtagcccctttgactactggggccaaggccaggtcaccgtctcctca

SEQ ID NO: 35 - protein, 108 aa, artificial sequence
  protein
DAVMTQTPLSLPVSLGDQASISCRSSQSLENSNGNTYLNWYLQKPGQSPQLLIYRVSNRFSGVLDRFSGSGSGTDFTLKISRVEAEDLGVYFCLQVTHVPPTFGAGTK

SEQ ID NO: 36 - DNA, 324 bp, artificial sequence
  DNA
gacgctgtgatgacccaaactccactctccctgcctgtcagtcttggagatcaagcctccatctcttgcaggtctagtcagagccttgaaaacagtaatggaaacacctatttgaactggtacctccagaaaccaggccagtctccacagctcctgatctacagggtttccaaccgattttctggggtcctagacaggttcagtggtagtggatcagggacagatttcacactgaaaatcagcagagtggaggctgaggatttgggagtttatttctgcctccaagttacacatgtccctcccacgttcggtgctgggaccaag